European Patent Specification EP 3 923 713 B1, published November 19, 2025. Title: TRANSGENIC MOUSE MODELS SUPPORTING INNATE IMMUNE FUNCTION. Applicant: The Jackson Laboratory. Application Not yet assigned. The sequence listing filed with the application follows.

SEQUENCE LISTING (7 sequences)

SEQ ID NO: 1 - RNA, 19 nt, Artificial Sequence
  Synthetic polynucleotide
gaacagcuuggugcauucg

SEQ ID NO: 2 - RNA, 19 nt, Artificial Sequence
  Synthetic polynucleotide
gauggucaccaacgcugac

SEQ ID NO: 3 - DNA, 24 bp, Artificial Sequence
  Synthetic polynucleotide
ccaacctgaactgtatggagatag

SEQ ID NO: 4 - DNA, 20 bp, Artificial Sequence
  Synthetic polynucleotide
ccacagggaaagccactaaa

SEQ ID NO: 5 - DNA, 1500 bp, Mus musculus
atcccccagtgctggtgaccttgaacacagggtctgccctgagcagtgctgacagcctgttagctgtcattttgaagcatttcctgaaggaaacttaccttatcattgcagctgtaaagaagaaggccctgctgttgtcagaaaggaggaaaaggtacttcatgagttgttcggaacagacatcagatgctgtgctagaaatgcactgggccgcgaatgcaccaagctgttcaccataggtaatgggggactgtcggctatgtgtccttagtgacggttcctaagggaccggtgatagcttctgtgtgggtaatcattccacttcagaaagatgatggaaagttatactgaaatccgaatctagatcgaatagtccacattctgacataaaagcaattgaacacacaggtatggccaagcttggtggcccgggcttttaatccttctttcataggactttgatttgattcaatttgatttgatttgatttgacttaggtgctgggctcaaacccagggactcagagcatctgctttgccactgagttccactccagatcttttgcaccactttatttatttatttattgtgtgtgtgtatacacacattaaatacacacacatacacacacacacacacacacacacacacacacacacacacacacacacacgctacagcatgtaatgtggatgtcaggttctcttcttgtcatatggggcccctggatcaaattcaggtcagtctggcagcggcaggcacctccacccactgagccatcttgatgccccgttcataccatttacaatgtaacactgtagattctgtaagggaggatttctgcaacaaagggtattccatctcgagtgggtggttttactctgtcgcttttttttttttagttttgtgctgctctgtgactccaggtcttctccaggccagcctcttttaccctgatcttctcagctctgcattgtttggcttgattagtgatggcagggatgctgacaccattgcttttcaaaacgtttgcgacacttctgagctgaggcaaaagtttttaaaaaaaagatgtgcttttttttttttttttttgtcttctttgggatatttttatcttctagatctaaaccaggctcctcagagcacactgccccagttattcctgaaagtgggggaacccttgtggatcaggtgtaaggccatccatgtgaaccatggattcgggctcacctgggagctggaagacaaagccctggaggaggtaacagcgcccacccgtggtgtttaccgtaagctctcagcgtgggctggaaacccggaatacagactcccctttcattaatactcagggcagctactttgagatgagtacctactccacaaacaggaccatgattcggattctcttggcctttgtgtcttccgtgggaaggaacgacaccggatattacacctgctcttcctcaaagcaccccagccagtcagcgttggtgacca

SEQ ID NO: 6 - DNA, 442 bp, Artificial Sequence
  Synthetic polynucleotide
ccaacctgaactgtatggagatagcttgtctatggggaaaaaaaatcaccaaataaaataaaatctaaaatattaaataataaagtaatactgtaacattatcctaattagatacagagtagctagctggtccctgcagattccaggctggatacagttgagttaatttttcatctgctcttttcttccatccctaaaaatatactttgtaacttcatcccctaaacatactgggtccccccaccccatcctaggtaacgggctcacgaaatttggggttggttggtttgtttgtttttaatgctgtcctggaactcgctgtgtagattggttggccttgaactcacagaaatctaccagcatctgcctccccagtgctgggattaaaggcacaggccaccaagcttgactctgcttgtgtctttagtggctttccctgtgg

SEQ ID NO: 7 - DNA, 13880 bp, Homo sapiens
gatccctgtgctcctccgagtggcacaggaaacttggctgatagaggcgctctctccatgcatcctccaccatccactccccggtcccttagacttccattcagaagtgacacctgtcacctccaccctcatgtgactggccaaagtgagtgtggccatgtccgagttccccaggatgggacctcgaatcctcctgctgggggggtgggggcagcagatgtttcaggacagtctgccacggatcagatgggtgagcaagagattcaggatgggcgtgatgggtcacacctgtaatcccagcattttgggaggccgaggcaggctgatcacctgaggtcaggagttcgagatcagcctggccaacatagtgaaacctcgtctctactaaaaatacaaaaattagccgggcatggtggcacgcacctgcaattccagctacttgggagcctgaggcacaagaattgcttaagcccaggaggcggaggttgccgtgagccgagactgtgccactgcactccagcctgggcaacagagtgagaccccatctaaaaaaaaaaaatgcttcagagattcagagatccacagatgtggaagagagcttctattttgtctcatgtaccacctcacccctcagtttggagttggagaagccgaggcttagagaggtcaaggggctggccaagctcccacagtgataaagctagtgctagggcgacacctgccaggcccaatgtgacaagatgcatcctgagtcctgtgtgccaagccttggcggggcaaagttggggcccggaggacggtaagacacagcaactgcgagttcccagagacagatccgggttccagccccagctcaccatgcactgggcgtgccacccagggagtcagccccactgcagcccccgctgcggggcgtccggagaacgcgccatctgcggcgtgagcggccgcctctcaccaccagggggcgcgctccgcctgggcccagattccaccccttgactgtctccccccaaaaatttcctttcactttcggtctctggctgtcacccggcttggccccttccacacccaactggggcaagcctggtgcgtgaggagacttggactctaggtccccaaggggcggagccagggtccccactcctggggcagggggagcagagggtggggggctgggttcccgggtccctaacctggggagggttctggggaccagacgtcgaggttcttagaagtggagatgaagagttttcaccgtaactggggcagacgcaggaagcctgggggaggaaggggcggaaactcagccacatcaatgggacgcgggaggggcggggaggcaaaggggcgggcagggcaggggctggggcatgagggtccgagacttgttcttctgtcccttccaagacccggcgacaggaggcatgaggggcccccggccgaaatgacagtgctggcgccagcctggagcccaacagtgcgtaaaccccagggacaagatcaggggagaggggaggcacaatgtcaggatggggcagagatgaggggagatggacgggagaacagatggacagatgacgaggaaataggaggggagatggacagatgtgaggggagatggataggagaggagacggacagaggagggggagatggacagaggatggggagatggacagaggagggggagatagaggagagggagatagagaggagtgggagatggacaggagcggggagatggacagaggagggggagatggacagaggagagggcagatgaacagaggagagggagataaagaggagggaggtggacaggaggagggagatggacagagaagggggagatggacagaggtgggggagatggacaggagggaagatggagaggagggggtatggacagaggagaggggagatggacaggagggggagatggacagaggagagggagatgaagaggagggggaggtggacaggaggagggagacggacagaggagaggaagagagacagaggaggggggagatggacagaggagggggagatggacagaaaaggggggagatggacagaggagagggaaggtggacagagccaagaacaaatgaagaggacgtggaccaagatcaagagagaagcaggcaacagtggtgtagaaggcagagggagggacagagctggaggaacccgggcgaggaaaccagacgtgaagatgaggtggttggagagagaccagcagagtgggggagatggggagagagaggggtggggcagagggggatgcaaactggacagcattggaccagaggcagagagaaaccgggaaagacaggcagagatggggccatgtctccagaaagtgtggaagaggcagaaggacacccagggaaggaggagcggggaagacagaacagtacaggtgggaagcccggaggagggggctgtgtgtggaacagcagagggctcccccagcacccgctcccctgcagacctatctcctcctgctgctgctgctgagctcgggactcagtgggacccaggactgctccttccaacacagccccatctcctccgacttcgctgtcaaaatccgtgagctggtgagcggcgctgccccggaccccctcatgtgatcccccttccccccacttttttttttaagtagagatggggtctctctccctgtgtttcccagggtggtcttgaactcctgggctcaagcgatcctcccaccttggcctcccaaagtgctggaattacaggcgtgagccactgtgcttaggggtgtcatccctttttaagggcaaggttctgtggcttcttctgggctccccctctcttggtcttgtccctctctctctggatctctgctgccacctctgggtccccacagttctgtttctcgctgttttcagccaggcctgatcctgttttctcccgcagtctgactacctgcttcaagattacccagtcaccgtggcctccaacctgcaggacgtaagtcatgttgggagggacctgggatggaggtggggaccacagactcaagatgctccaccgaggcgagtggataaccaggccctcccctccccaaacccaggaatcagagtcctcagcccctcctccctcagacccaggagccccggcccagcccctcctccctcagacccagcagccccgtgcccagctcctccctcagacccgtgggttctcccctctaggaggagctctgcgggggcctctggcggctggtcctggcacagcgctggatggagcggctcaagactgtcgctgggtccaagatgcaaggcttgctggagcgcgtgaacacggagatacactttgtcaccaaatgtgcctttcaggtcagccctcaacttaggggacaagtgaggggagggagatgccttcctacgaattagaagtaaagctccactaggccttattggcgatttggaccatagccacccaacgaaggtagagcgagaagcgccaccctgcagagccctgttcctacagaacaacacgtccccaggcaccggtgatggggagcagtctggtcccattctggggccccggtttcctaggccatgatgaagggtgccactgaggggttcttcccccaaaaaaaaacagggagagaaggggtctctaaactgaggaggccgggcgtggtggctcactcctgtaatcctagcactttgggaggctgaggtgggcggatcacttgaggtcaggagtttgagaccagcctggccaacatgatgaaatcccggctgtactaaaaatacaaaaattagccgggcatggtggctcaggaggctgaggcacaggaatcgcttgaacccgggagccagaggctgcagtgagccgagatcatgccactgcactccagcctgggagacagagtgaaactgtctcaaaaacaaaacaaacaaacaaaaacctctctctgagggctgggtgcagtggctcacacctgtaatcccagcactttcggaggccaaggtgggaggattatttgagcccaggagttcaagaccagcccgggtaacacagtgaaacctcatctctgcacaaaaataaaaataaattagccaggcatggtggtgcccacctgtggtcccagctactcagaaggctgaggtgggaggatcacttgagccctggaggtcgaggctgcgatgagctatgattgggccactgcactccagcttgagcgacagagcaagaccctgtctcaaaacatagaataggccgtgtatggtggctcacgactgtaatcccagcactttgggaggctgaggcgggtggattgcctgagctcaggagttcgagaccagcctcggcaacgtgatgaaaaccatctctactaaaatacaaaaacaaaattagccaggcatggtggtgggcacctgtagtcccagctacttgggagactgaggcaggagaattgcttgaacccaggaggcagaggttgcagtgagccgagatcacaccactgccctccagcctgggcgacagagcaagactccatctccaaaaaaataaaaataaaataaaagcctgggtacagtggctcacgcctgtaatcccagcactttgggagcccgaggcgggcagatcacgaggtcaggagtttgagaccaccctggccaatgtggtgaaaccccgtctctactaaaaatacaaaaattagctgggcatggtggcgcgcgcctgtagtcccagctactcaggaggctgaggcagaattccttgaacccgggaggtagaagttgcagtaagccgagatcgtgccactgtactccagccagggtgacagagcaagactctgtccccaaaaaataaataaataataaagtaactttgggaggccgaggcgggcgagtcacctgaggtcaggagttcgagaccagcctggccaacatagagaaaccccgtttctactaaaaaatataaataaataaataaataaataaataggctgggcacggtggctcacgcctgtaatcccacactttgggaggccgaggcgggcggatcacaaggtcaggagatcaagaccatcctggctaacacaatgaaaccccatctctactaaaaatacaaacaattagccgggcgtggtggcaggcgcctgtagtcccaactacctgggaggctgaggcaggtgaatggcgtgaaaccaggaggcggagcttgcagtgagccgagattgcgccactgtactccagcctgggcaacagagcgagactctgtcttaaaaataaataaataaataaatatggccaagcacggtggctcatgcctacaatcccagcactttgggaggccaaggtgggcagatcacctgaggtcaggagttcgagaccagcctggccaacatggagaaaccccgtctctactacaaatacaaaaaatagctgggcatggtggtgggcacctatagtcccaaccactgaggaggctgaggcaggagaatcacttgaacctgggaggcagaggttgcatttcaccactccagcctgggcaacagagtgagactctatctcaaaaaaaaattaattaattaaataaataaactctgagagccagagctcactgggccctgttgctgggcatcgccagcagggaagggcctttggcctgcggaggggcggtggggggatgacgtggtggtgacgtctccctcccctgctcccagcccccccccagctgtcttcgcttcgtccagaccaacatctcccgcctcctgcaggagacctccgagcagctggtggcgctgaagccctggatcactcgccagaacttctcccggtgcctggagctgcagtgtcagcccggtaaaggcttccaggcacccccactccttcccctcctgtcctcacggccgctcctcctctctgcacagtgcatcccagaccccatctttctcatattggttgtgacaagggcaagcttattcctctttctggagctcagtttaccaattttttttttttttttttgagacggagtctcgcactgtcgcccaggctggagtgcagtggcgtgatcttggctcactgcaagctccgcctctcgggttcatgccattctcctgcctcagcctcccaagtagctgggaccacaggcgcccgccaccacacccggctaattttttgtatttttagtagagacggggttttaccgagttaaaccaggatggtctcgatctcctgaccttgtgatccacctgccttggcctcccaaagtgctgggattacaggcgtgagccacagtgcccagcctacctttttttttttttttttttttgagatggagtcttgctctgtcccccaggctggagtgcaggggtgctatctcggctcactgcaagctctgcctcctgggttcacgccattctcttgcctcagcctccccagcagctgggactacaggcgcctgccacctcacgcggctaatttttttttttgtatttttagtagagacggtgtttcaccgtgtcagccaggatggtctcgatctcctgacctcgtgatctgcccgcctcggcctcccaaagtgctaggattacagatgtgagccaccgcgcccagcctattgttttttttttctaagtcggagtcttgctctgtcgcccaggctggagtgcagtggcgcaatcttggctcactgcaacctccatctccagggttcaagcgaatcttctgcctcagccttccgagtacctgggattacagatgcgcataccatgcctggctagtttttgtgtttttagtagagatgggttttcaccatgttggccaggctggtcttgaactcctgacctcaagtgatccacccaccttggcctcccaaagtgctgggattataggcgtgagccaccgcgctcagcctattcactcatttaatttgtgacagtctgatgaggtaggtacaatgattatcctagttttacagatgagcaaactgaggcacagagaggccaagcagcccatccaaggtcacacagccagtggcagccaggcctctctttccttccttaccccagcccttctccttggtcacccagcctcctctttctccccagactcctcaaccctgccacccccatggagtccccggcccctggaggccacagccccgacagccccgcagccccctctgctcctcctactgctgctgcccgtgggcctcctgctgctggccgctgcctggtgcctgcactggcagaggacgcggcggaggacaccccgccctggggagcaggtgagcaggctgggaagagggggtgagggggccgagagggtggcccacttgtggctgacactttggggcccacaggtgccccccgtccccagtccccaggacctgctgcttgtggagcactgacctggccaaggcctcatcctggtgagtccttcctgggctatggggcctggactttgtgtctgcaggttgggagggtcactaggaggccatggaagggtggtgagcagtggaggggcaggggcagctctaggtgcagaaagacccctctggggccaggcgcggtggctcacgcctgtaatcccagcactttgggaggccgaggcgggtggatcacttgaggtcaggagttcaagaccagcctggccaacatggcaaaccccagtctctactaaaaatacaaaaattaactgggcatagtggtgtgtgcctgtaatcccagctactcaggaggctgaggaaggagaattgcttgaacccaggaggcggaggttgcagtgagccgagattgcgccactggactccagcctgagtgacagagctagactccgtctcaaaaaaaaaaaaaaaaaagaaaaggaaagacccctctggggccacggagacagactggagaccaagccggaggctgtgggaaggcccagggtgaggaccatgactgagccagggctgggaccatgggatggagtggagtggatgggcagagagtcaggggtcagagatcaggagggaccggcctggggcctgacaggcttgagttggcacagatagccctggtccagtgatggggtggacaggggggaacctgggggaggagtcagattagggaaagacatggagctcactggggacctgaaggagcaaggggccctggggagatctgtggatgtgggagtttgcaagcctcctgggacaggaaggaaatggcattccagaaagagggaactgcctttggaagccctttggtatgagaaagctcagggtgttccagtaacttgggccagcgtggggcagcaaggagccatgggaggtgtgagagggaggaaaggagctgggaacaggtgtggagggtgcaggcaggtaggcaggtgggccaggagggaagaaggaggggaggccccagcgggtcccctaacatttcaaatctaacattttgtagtaattgctcgcacatatagtgccttggtaatgcaggcctcatgtggggctggcttgcttgctttatttttttttgagatggactctcactctgtcacccaggctggagtgcagtggcgggatcttggctcactgcaacctccacctcccaggttcaagcaattctcctgcctcagcctcccaagtagctgggattacaggcgcccgccaccatgcctggctaattttttgtatttttagtagagatggggtttcgccatgttggccaggctggtctcaaactcctgatctcagctgatccgcccgcctcagcctcccaaagtgctgggatgacaggtgtgagccactgttcctggcccatgctgggctttccacaaatgaactcacttccttgagaagttcgtgccattatgatcccaaggcatagagaggtaaataatttgccaaaagtcacacagctcaagggtgacaaccaagatttgacttcaggttgtcttttttttttttttgagatggagtcttgctctgtcgcccaggctgtagtgcagtggcatgatctcggctcactgcagcccccgcctcccaggttcaagtgattctcctgcctcagcctctggagtagctgggattacaggtacccaccaccacactcggctaatttttgtatttgtagtagagacggggtttcaccatgttggccaggctggtctcgaactcctgaccttagctgatccgcccgcctcagcctcccaaagtgctgggattacaggcatgagccaccacgcccggcctcgagtttgtcttgatccagcatctgtgcccttcactctgctgcctcagtttcctgatctgtacaaaaggctctaataatagtccttccaccatagggttgttatggggtgaagtgaagtgacacaggcaaggctcttagagcaacgcagtggaaacggcatgtgagccacctgtgcgattttcactttcctggtagccacattttttttttttttttcctgagatggagtctcactctgtcgccaggttgaagtgcagtggtgtgatctcagctcactgcaacctccacctcccgggttcaagcgattctcctgcttcagtctaccgagtagctgggattacaggcacgcgccatcacgcccggctaattttttgtgtttttagtagagacaaggtttcaccatgttggtcaggctggtctcgaactcctgacctcatgatccacccgcctcagcctcccaaagtgctgggattacaggcgtgagccaccgcgcccggggtcacagtttttaaaaaaggaaaaagaagcaggtaactttattttatgcagtatatccaaaatgttgttatttcaacatgtaatcagtatttctcaatgattaatgagacattaatcagttggaatcattcatcattttgggatattttacattcttttgtcatactaagccttcagcatccaacgtatagtttatttatttatttatttttccttttgagatggattctcgctctgtcacccaggctggagtgcagtggcgcgatctcagctcactgcaacctcggactccctggttcaggcgattctcctgcctcagcctcccgagtacctgggattacgccaccacacccagctaatttttgtacttttagtagagaccgggtttcaccatgttggccaggatgatctccatcccctgacctcgtgatccgcccgcctcagcctcccaaagtgctggattacaagtgtaagccaccgcgcccagcccagacaataaatttttatcagaaatgcttcatctatatttaaatttcatgaaatttacagttgccaaaagtagactcacatagtcaagttgttcaaaacatacattaaaccagcctgggccacatggtgaaaccccatctctacaaaaaattttaaaaagtagctgggtgtggtggcacatgcctgcagtcccagctacttaggaggcaaagtaggaggattgcttgagcccaggaggtcgaggctgcagtgagccctgattgtgccactgcactccagcctgggtgagagagcaagaccctgtctcaaaaacaaaaaaaccacacagaagagtttagaatcccagttgctatctctgggaatcatcatgattgctaagaccggtatctatccaacaacaacaaaaataattagtgcactccagcctgggcaatagagggagactctgtctcaaaaaaaaaaaaaaaaaaaaaaaaaagatcaaagaccagtatctaaattgctctgtcgcccagggtggagtgcagtggcacgatctcggctcactgcaacctccgcctcccgggttcaagtgattctcctgcctcagcctccccagtagcttggactacaggcgcgtgccaccacacccagctaatttttgtatttttagtagaggtagggtttcactatgtttgccaggattgtctcgatctcttgacctcgtgatctgcccgcctcagcctcccaaagtgctgggattataggcgtgagccaccacgcccagcctatctttttttttttttttaagaaaaggtaatacattgagcagttttcctcccaacctagtccctgtccaatctgtttcctgtcttaaatttattttttattataatttttttttttttttttttttgtgagacagacttttgctcttgttagccaggctggagtgcagtggtgctatcttgactcacggcaacctccacctcccaggttcaagcgattctcctgcctcagcctctggagtagcttggattacaagcgcctgccaccacgcccaactaatttagtgtatttttagtagagacggggtttcttttgttgttgttgttgtttttgagacggagtctcactctattgcccaggctggagtgcaacggcacgatctcggctcactgcaacatctgcctcccgggttcaagcgattctactgcctcagcctcctgagtagctgggattacaggcacacaccaccacacctggctaatttttgtatttttagtagagatggggtttcaccatattggccaggctgatctcgaactcctgacctcgtgatctgcccgccttgacctcccaaagtgataggattacagccatgagccgccctgcccaactaatacctgatattaattttattgtatctcacccagcatggtggctcacacctgtaactccttggcagatcgcttgagcctaagagttcaagaccagcttgggcaacatggtgaaaccccgtctctactaaaaatataaaaatgagctgggcatggtggcgtgcacccgtaatcccagctaactcaggaggctgaggcaggaagaatggcttgaacccgggaggcagaggctgcagtgagctgagatcatgccactgcattccagcctgaaacagagcaagactgtctcaaaagaagtttaagtccagcctcaaactcctggactcaagtgatcctcctgcctcagcctcctgagtagtgcaccggccccatctcaagtgttcagtattcacatgtggcttgttactcccgtattaaagagcaaaaatagagaacgtttctttttcttttttttctttttttttttttttttgagatgggagtttcgctcttgtcgcccaggctggagtgcaatggcacgatcttggctcaccgcaacctctgcctcccaggttcaagcgattctcctgcctcagcctcccaagtagctgggattacagacatgcaccaccatgcctagcaaattttgtttttgtttttgtttttttcttttgagacagacttttgcttttattgccaaggctggagtgcaatggtgcaatctcgactcactgcaacctccgcctcccgggttcaagcaattctcctgcctcagctaattttgtagttttagtagaaacggtttctccatgttagctaggctggtctcaaactcccaacctcaggtgatccgcccgcctcgacctcctaaagtgctggaattacaggcgtgagccactgtgcctggccctaattttgtatttttagtagagatggggtttctccctgttggtcaggctggtctcaaactcccaacctaaggtgatccaccagcctcagcctcccaaactgctgggattataggcatgagccaccgcgcccggggaaatatagggaacatttctatcatggccacgttctcttggacagcaatgccctagcacatagtaagcgcttgctgggaatggagttgttttgggcataaatctgtggcccgccccaagctaagctactttccctctcctctctcagcggagccttaaacaacgcagtgagacagacatctatcatcccattttacaggggaggatactgaggcacacagaggggagtcaccagccagaggatgcatagcctggacacagaggaagttggctagaggccggtcccttccttgggcccctctcattccctccccagaatggaggcaacgccagaatccagcaccggccccatttacccaactctgtacaaagcccttgtccccatgaaattgtatataaatcatccttttctaccagctctggccaggtctgtctatggatgggtgtgaatggggtagttttgatttcagaatcttggtttttgaattgcaatgcaatgtttcattcaatacgtgttttctgaggtcccctggagccccgggccggcgctgggcaatgtcagagcctggatttgagtcagaaccagcccaggtgccccaggtctccttggctatggacgagaagacaagggattcagcgagcctgggtgcaggatgccataggctactatggagataaaacagaggcagtgtgaggggcaactcacccaggcagggagagcagagaggctttccagagccaaatggcattgcgatggtgacaagccagatttggagggggtggggagggcatcctgggcaagggacccagctgaagcaaaggccgacagtccagaaagtgagaagttcctctgaggaacgctcagtggattggtgcagccaggcaactagaagccattccttgatccactcttagagcccctggggaagaccacctccatctgttttacagatggataaactgaggcccagataaggccaagggtttctccaggtcacagtgaagtcgaccagacacaggaatccaaatctctaagcctagaatgggcaaggctccggggctcacgccggtaatcccagcactttgggaggccgaaacgggaggatcgcttgagcccaggagttcgagatcagcctggccaacatgtcagactccccccgttcccgggccacaacaaaatatatatatatatatatattagccaggcatggtggcgcgcccctgtagtccaagttactcgagaggctgaggcaggag